European Patent Specification EP 3 597 746 B1, published April 19, 2023. Title: A method for producing an RNA molecule-peptide complex and use thereof. Applicant: RIKEN. The sequence listing filed with the application follows.

SEQUENCE LISTING (23 sequences)

SEQ ID NO: 1 - protein, 21 aa, Mus musculus
MEVGWYRSPFSRVVHLYRNGK

SEQ ID NO: 2 - DNA, 66 bp, Artificial Sequence
  random library DNA
  misc_feature (19)..(42): n is a, g, c or t ; m is a or c
gctgccgctgccgctgccmnnmnnmnnmnnmnnmnnmnnmnncatatgtatatctccttcttaaag

SEQ ID NO: 3 - DNA, 50 bp, Artificial Sequence
  primer
cctaatacgactcactatagggttaactttaagaaggagatatacatatg

SEQ ID NO: 4 - DNA, 39 bp, Artificial Sequence
  primer
  modified_base (1)..(2): gm
ggtcggcggatcaaagtagctgccgctgccgctgccgca

SEQ ID NO: 5 - DNA, 113 bp, Artificial Sequence
  random DNA library
  misc_feature (51)..(74): n is a, g, c or t ; k is g or t
cctaatacgactcactatagggttaactttaagaaggagatatacatatgnnknnknnknnknnknnknnknnktgcggcagcggcagcggcagctactttgatccgccgacc

SEQ ID NO: 6 - DNA, 16 bp, Artificial Sequence
  Pu-DNA
ctcccgccccccgtcc

SEQ ID NO: 7 - DNA, 23 bp, Artificial Sequence
  splint DNA
gggcgggagggtcggcggatcaa

SEQ ID NO: 8 - DNA, 39 bp, Artificial Sequence; identical to SEQ ID NO: 4
  primer

SEQ ID NO: 9 - DNA, 20 bp, Artificial Sequence
  primer
ccgaaggagatatacatatg

SEQ ID NO: 10 - DNA, 19 bp, Artificial Sequence
  primer
  misc_feature (2)..(3): n is a, g, c or t
annctgccgctgccgctgc

SEQ ID NO: 11 - DNA, 107 bp, Artificial Sequence
  Flag DNA
ggcgtaatacgactcactatagggttaactttaacaaggagaaaaacatgaagtactccccaaccgactgcggcagcggcagcggcagctactttgatccgccgacc

SEQ ID NO: 12 - DNA, 140 bp, Artificial Sequence
  Template DNA 1
cctaatacgactcactatagggttaactttaagaaggagatatacatatgaagtactccccaaccgactgcaagaaggactacaaggacgacgacgacaagtgcggcagcggcagcggcagctaggacggggggcggaaa

SEQ ID NO: 13 - DNA, 140 bp, Artificial Sequence
  Template DNA 2 & 3
cctaatacgactcactatagggttaactttaagaaggagatatacatatgaagtactccccaaccgactgcaagaaggactacaaggacgacgacgacaagtgcggcagcggcagcggcagctactttgatccgccgacc

SEQ ID NO: 14 - protein, 8 aa, Artificial Sequence
  peptide derived from random DNA
KSPFSRLT

SEQ ID NO: 15 - protein, 6 aa, Artificial Sequence
  peptide derived from random DNA
RSPFNR

SEQ ID NO: 16 - protein, 8 aa, Artificial Sequence
  peptide derived from random DNA
YSSPFNRK

SEQ ID NO: 17 - protein, 8 aa, Artificial Sequence
  peptide derived from random DNA
HRSPFNRK

SEQ ID NO: 18 - protein, 8 aa, Artificial Sequence
  peptide derived from random DNA
ISEYKLRL

SEQ ID NO: 19 - protein, 8 aa, Artificial Sequence
  peptide derived from random DNA
KSPFSRLT

SEQ ID NO: 20 - protein, 8 aa, Artificial Sequence
  peptide derived from random DNA
SPFSRLTC

SEQ ID NO: 21 - protein, 8 aa, Artificial Sequence
  peptide derived from random DNA
YRSPFNRK

SEQ ID NO: 22 - protein, 8 aa, Artificial Sequence
  peptide derived from random DNA
KSPFSRLT

SEQ ID NO: 23 - protein, 8 aa, Artificial Sequence
  peptide derived from random DNA
SPFSRLTS